European Patent Specification EP 3 268 028 B1, published May 21, 2025. Title: Compositions and Methods for Treating Cancer. Applicant: Rush University Medical Center. The sequence listing filed with the application follows.

SEQUENCE LISTING (44 sequences)

SEQ ID NO: 1 - DNA, 20 bp, Artificial Sequence
  Artificial mouse IFN gamma primer, sense strand
cggcacagtcattgaaagcc

SEQ ID NO: 2 - DNA, 20 bp, Artificial Sequence
  Artificial mouse IFN gamma primer, antisense strand
tgcatcctttttcgccttgc

SEQ ID NO: 3 - DNA, 20 bp, Artificial Sequence
  Artificial mouse IL10 primer, sense strand
taaggctggccacacttgag

SEQ ID NO: 4 - DNA, 20 bp, Artificial Sequence
  Artificial mouse IL10 primer, antisense strand
gttttcagggatgaagcggc

SEQ ID NO: 5 - DNA, 20 bp, Artificial Sequence
  Artificial mouse Tbeta primer, sense strand
attggttggagaggaagcgg

SEQ ID NO: 6 - DNA, 20 bp, Artificial Sequence
  Artificial mouse Tbeta primer, antisense strand
tgtgcacccttcaaaccctt

SEQ ID NO: 7 - DNA, 20 bp, Artificial Sequence
  Artificial mouse GATA3 primer, sense strand
tggcgccgtcttgatagttt

SEQ ID NO: 8 - DNA, 20 bp, Artificial Sequence
  Artificial mouse GATA3 primer, antisense strand
cctcttccgtcagcggatac

SEQ ID NO: 9 - DNA, 20 bp, Artificial Sequence
  Artificial mouse Foxp3 primer, sense strand
tgtgcctggtatatgctccc

SEQ ID NO: 10 - DNA, 20 bp, Artificial Sequence
  Artificial mouse Foxp3 primer, antisense strand
gttcttgtcagaggcaggct

SEQ ID NO: 11 - DNA, 20 bp, Artificial Sequence
  Artificial mouse GAPDH primer, sense strand
gcatcttcttgtgcagtgcc

SEQ ID NO: 12 - DNA, 20 bp, Artificial Sequence
  Artificial mouse GAPDH primer, antisense strand
tacggccaaatccgttcaca

SEQ ID NO: 13 - DNA, 20 bp, Artificial Sequence
  Artificial mouse PDL-1 primer, sense strand
tcacttgctacgggcgttta

SEQ ID NO: 14 - DNA, 20 bp, Artificial Sequence
  Artificial mouse PDL-1 primer, antisense strand
tgccaatcgacgatcagagg

SEQ ID NO: 15 - DNA, 20 bp, Artificial Sequence
  Artificial mouse PDL-2 primer, sense strand
ggtgtgtgattggtaggcca

SEQ ID NO: 16 - DNA, 20 bp, Artificial Sequence
  Artificial mouse PDL-2 primer, antisense strand
catccagcaggtaaccaggg

SEQ ID NO: 17 - DNA, 20 bp, Artificial Sequence
  Artificial mouse PD-1 primer, sense strand
atctacctctgtggggccat

SEQ ID NO: 18 - DNA, 20 bp, Artificial Sequence
  Artificial mouse PD-1 primer, antisense strand
gagtgtcgtccttgcttcca

SEQ ID NO: 19 - DNA, 20 bp, Artificial Sequence
  Artificial mouse CTLA-4 primer, sense strand
tactctgctccctgaggacc

SEQ ID NO: 20 - DNA, 20 bp, Artificial Sequence
  Artificial mouse CTLA-4 primer, antisense strand
ccgtgtcaacagctctcagt

SEQ ID NO: 21 - DNA, 20 bp, Artificial Sequence
  Artificial mouse Cytochrome C primer, sense strand
cccccagcctcccttatctt

SEQ ID NO: 22 - DNA, 20 bp, Artificial Sequence
  Artificial mouse Cytochrome C primer, antisense strand
ggtctgccctttctcccttc

SEQ ID NO: 23 - DNA, 20 bp, Artificial Sequence
  Artificial mouse Caspase 3 primer, sense strand
gagcttggaacggtacgcta

SEQ ID NO: 24 - DNA, 20 bp, Artificial Sequence
  Artificial mouse Caspase 3 primer, antisense strand
ccgtaccagagcgagatgac

SEQ ID NO: 25 - DNA, 21 bp, Artificial Sequence
  Artificial mouse Caspase 8 primer, sense strand
aacattcggaggcatttctgt

SEQ ID NO: 26 - DNA, 21 bp, Artificial Sequence
  Artificial mouse Caspase 8 primer, antisense strand
agaagagctgtaacctgtggc

SEQ ID NO: 27 - DNA, 20 bp, Artificial Sequence
  Artificial mouse Caspase 7 primer, sense strand
ttttcccaaagctgccctcg

SEQ ID NO: 28 - DNA, 20 bp, Artificial Sequence
  Artificial mouse Caspase 7 primer, antisense strand
gcgtcaatgtcgttgatggg

SEQ ID NO: 29 - DNA, 20 bp, Artificial Sequence
  Artificial mouse Caspase 9 primer, sense strand
ctctgaagacctgcagtccc

SEQ ID NO: 30 - DNA, 20 bp, Artificial Sequence
  Artificial mouse Caspase 9 primer, antisense strand
ctgctccacattgccctaca

SEQ ID NO: 31 - DNA, 20 bp, Artificial Sequence
  Artificial mouse P53 primer, sense strand
accagggcaactatggcttc

SEQ ID NO: 32 - DNA, 20 bp, Artificial Sequence
  Artificial mouse P53 primer, antisense strand
agtggatcctggggattgtg

SEQ ID NO: 33 - DNA, 20 bp, Artificial Sequence
  Artificial mouse BAD primer, sense strand
cagcgtacgcacacctatcc

SEQ ID NO: 34 - DNA, 20 bp, Artificial Sequence
  Artificial mouse BAD primer, antisense strand
cgggatcggacttcctcaag

SEQ ID NO: 35 - DNA, 20 bp, Artificial Sequence
  Artificial mouse BID primer, sense strand
tctgaggtcagcaacggttc

SEQ ID NO: 36 - DNA, 20 bp, Artificial Sequence
  Artificial mouse BID primer, antisense strand
tttgtcttcctccgacaggc

SEQ ID NO: 37 - DNA, 20 bp, Artificial Sequence
  Artificial mouse BAX primer, sense strand
ctggatccaagaccagggtg

SEQ ID NO: 38 - DNA, 20 bp, Artificial Sequence
  Artificial mouse BAX primer, antisense strand
cctttccccttcccccattc

SEQ ID NO: 39 - DNA, 20 bp, Artificial Sequence
  Artificial mouse BCL2 primer, sense strand
agcatgcgacctctgtttga

SEQ ID NO: 40 - DNA, 20 bp, Artificial Sequence
  Artificial mouse BCL2 primer, antisense strand
gccacacgtttcttggcaat

SEQ ID NO: 41 - DNA, 20 bp, Artificial Sequence
  Artificial mouse BCL-XL primer, sense strand
ttgtacctgcttgctggtcg

SEQ ID NO: 42 - DNA, 20 bp, Artificial Sequence
  Artificial mouse BCL-XL primer, antisense strand
cccggttgctctgagacatt

SEQ ID NO: 43 - DNA, 15 bp, Artificial Sequence
  Artificial mouse BAK primer, sense strand
cctgggccaacacgc

SEQ ID NO: 44 - DNA, 21 bp, Artificial Sequence
  Artificial mouse BAK primer, antisense strand
ctgtgggctgaagctgttcta